European Patent Application EP 4 596 578 A1, published August 6, 2025. Title: Monoclonal antibody and method for detecting A1 beta casein. Applicant: SOWAKAI SOCIAL MEDICAL CORPORATION. The sequence listing filed with the application follows.

SEQUENCE LISTING (227 sequences)

SEQ ID NO: 1 - protein, 10 aa, synthetic construct
  REGION 1..10: note = Part sequence of A1 beta casein
FPGPIHNSLP

SEQ ID NO: 2 - protein, 10 aa, synthetic construct
  REGION 1..10: note = Part sequence of A1 beta casein
FPGPIPNSLP

SEQ ID NO: 3 - protein, 19 aa, synthetic construct
  REGION 1..19: note = Part sequence of beta casein
ESLSSSEESITRINKKIEK

SEQ ID NO: 4 - protein, 8 aa, synthetic construct
  REGION 1..8: note = Part sequence of HCDR1
GFTFSNYG

SEQ ID NO: 5 - protein, 8 aa, synthetic construct
  REGION 1..8: note = Part sequence of HCDR1
GFTFSSYG

SEQ ID NO: 6 - protein, 8 aa, synthetic construct
  REGION 1..8: note = Part sequence of HCDR1
GFTFSNYD

SEQ ID NO: 7 - protein, 8 aa, synthetic construct
  REGION 1..8: note = Part sequence of HCDR1
GFTFRNYD

SEQ ID NO: 8 - protein, 8 aa, synthetic construct
  REGION 1..8: note = Part sequence of HCDR1
GYTFTTYT

SEQ ID NO: 9 - protein, 8 aa, synthetic construct
  REGION 1..8: note = Part sequence of HCDR1
GYTFTSYT

SEQ ID NO: 10 - protein, 8 aa, synthetic construct
  REGION 1..8: note = Part sequence of HCDR2
ISYDGSST

SEQ ID NO: 11 - protein, 8 aa, synthetic construct
  REGION 1..8: note = Part sequence of HCDR2
INYDGSST

SEQ ID NO: 12 - protein, 8 aa, synthetic construct
  REGION 1..8: note = Part sequence of HCDR2
ITTSGGST

SEQ ID NO: 13 - protein, 8 aa, synthetic construct
  REGION 1..8: note = Part sequence of HCDR2
ISPSGGSI

SEQ ID NO: 14 - protein, 8 aa, synthetic construct
  REGION 1..8: note = Part sequence of HCDR2
INPSSGYI

SEQ ID NO: 15 - protein, 8 aa, synthetic construct
  REGION 1..8: note = Part sequence of HCDR2
INPSSGYT

SEQ ID NO: 16 - protein, 8 aa, synthetic construct
  REGION 1..8: note = Part sequence of HCDR2
FNPSSGYT

SEQ ID NO: 17 - protein, 14 aa, synthetic construct
  REGION 1..14: note = Part sequence of HCDR3
ARPYNNYGYWYFDF

SEQ ID NO: 18 - protein, 18 aa, synthetic construct
  REGION 1..18: note = Part sequence of HCDR3
ARHGYYDGSYYYGGDFDY

SEQ ID NO: 19 - protein, 18 aa, synthetic construct
  REGION 1..18: note = Part sequence of HCDR3
ARHSYYDGNYYYGGSFDY

SEQ ID NO: 20 - protein, 9 aa, synthetic construct
  REGION 1..9: note = Part sequence of HCDR3
VRHGRRFDY

SEQ ID NO: 21 - protein, 8 aa, synthetic construct
  REGION 1..8: note = Part sequence of HCDR3
ARHRSFPY

SEQ ID NO: 22 - protein, 10 aa, synthetic construct
  REGION 1..10: note = Part sequence of HCDR3
ARHGHTQFAY

SEQ ID NO: 23 - protein, 11 aa, synthetic construct
  REGION 1..11: note = Part sequence of HCDR3
AVYDGYFPFDY

SEQ ID NO: 24 - protein, 11 aa, synthetic construct
  REGION 1..11: note = Part sequence of HCDR3
AGFAKDYPMDY

SEQ ID NO: 25 - protein, 6 aa, synthetic construct
  REGION 1..6: note = Part sequence of LCDR1
QNIYKN

SEQ ID NO: 26 - protein, 5 aa, synthetic construct
  REGION 1..5: note = Part sequence of LCDR1
SSVSY

SEQ ID NO: 27 - protein, 5 aa, synthetic construct
  REGION 1..5: note = Part sequence of LCDR1
SRVSY

SEQ ID NO: 28 - protein, 6 aa, synthetic construct
  REGION 1..6: note = Part sequence of LCDR1
QNINKY

SEQ ID NO: 29 - protein, 11 aa, synthetic construct
  REGION 1..11: note = Part sequence of LCDR1
QSLVHSDGNTY

SEQ ID NO: 30 - protein, 12 aa, synthetic construct
  REGION 1..12: note = Part sequence of LCDR1
QSLLNSRTRKNY

SEQ ID NO: 31 - protein, 8 aa, synthetic construct
  REGION 1..8: note = Part sequence of LCDR3
QQYYSGLT

SEQ ID NO: 32 - protein, 9 aa, synthetic construct
  REGION 1..9: note = Part sequence of LCDR3
QQWSNTPYT

SEQ ID NO: 33 - protein, 9 aa, synthetic construct
  REGION 1..9: note = Part sequence of LCDR3
QQWSSSPYT

SEQ ID NO: 34 - protein, 9 aa, synthetic construct
  REGION 1..9: note = Part sequence of LCDR3
CQHNSWPLT

SEQ ID NO: 35 - protein, 9 aa, synthetic construct
  REGION 1..9: note = Part sequence of LCDR3
FQHNSWPLT

SEQ ID NO: 36 - protein, 9 aa, synthetic construct
  REGION 1..9: note = Part sequence of LCDR3
LQSAHFPLT

SEQ ID NO: 37 - protein, 9 aa, synthetic construct
  REGION 1..9: note = Part sequence of LCDR3
QQSYNLPWT

SEQ ID NO: 38 - protein, 9 aa, synthetic construct
  REGION 1..9: note = Part sequence of LCDR3
KQSYTLPWT

SEQ ID NO: 39 - protein, 8 aa, synthetic construct
  REGION 1..8: note = Part sequence of HCDR1
GYTFTDHA

SEQ ID NO: 40 - protein, 8 aa, synthetic construct
  REGION 1..8: note = Part sequence of HCDR1
GFTFKNYG

SEQ ID NO: 41 - protein, 8 aa, synthetic construct
  REGION 1..8: note = Part sequence of HCDR1
GLTFRNYG

SEQ ID NO: 42 - protein, 8 aa, synthetic construct
  REGION 1..8: note = Part sequence of HCDR1
GFSFSNYG

SEQ ID NO: 43 - protein, 8 aa, synthetic construct
  REGION 1..8: note = Part sequence of HCDR1
GFTFSDYW

SEQ ID NO: 44 - protein, 8 aa, synthetic construct
  REGION 1..8: note = Part sequence of HCDR1
GFTFNNYW

SEQ ID NO: 45 - protein, 8 aa, synthetic construct
  REGION 1..8: note = Part sequence of HCDR1
GFTFSNYW

SEQ ID NO: 46 - protein, 8 aa, synthetic construct
  REGION 1..8: note = Part sequence of HCDR1
GYTFTNHY

SEQ ID NO: 47 - protein, 8 aa, synthetic construct
  REGION 1..8: note = Part sequence of HCDR1
GLTFSNYG

SEQ ID NO: 48 - protein, 8 aa, synthetic construct
  REGION 1..8: note = Part sequence of HCDR1
GLIFRNYG

SEQ ID NO: 49 - protein, 8 aa, synthetic construct
  REGION 1..8: note = Part sequence of HCDR1
GYTFTSNF

SEQ ID NO: 50 - protein, 8 aa, synthetic construct
  REGION 1..8: note = Part sequence of HCDR1
GFTFSKYD

SEQ ID NO: 51 - protein, 8 aa, synthetic construct
  REGION 1..8: note = Part sequence of HCDR1
GFTFSNFD

SEQ ID NO: 52 - protein, 8 aa, synthetic construct
  REGION 1..8: note = Part sequence of HCDR1
GFTFSTYD

SEQ ID NO: 53 - protein, 8 aa, synthetic construct
  REGION 1..8: note = Part sequence of HCDR1
GFTFDDYG

SEQ ID NO: 54 - protein, 8 aa, synthetic construct
  REGION 1..8: note = Part sequence of HCDR1
GFTFSDYY

SEQ ID NO: 55 - protein, 8 aa, synthetic construct
  REGION 1..8: note = Part sequence of HCDR1
GYTFTDYY

SEQ ID NO: 56 - protein, 8 aa, synthetic construct
  REGION 1..8: note = Part sequence of HCDR1
GSPLTSYT

SEQ ID NO: 57 - protein, 8 aa, synthetic construct
  REGION 1..8: note = Part sequence of HCDR1
GYTFSSYT

SEQ ID NO: 58 - protein, 8 aa, synthetic construct
  REGION 1..8: note = Part sequence of HCDR1
GYTFTTST

SEQ ID NO: 59 - protein, 8 aa, synthetic construct
  REGION 1..8: note = Part sequence of HCDR1
GYTFTDYS

SEQ ID NO: 60 - protein, 8 aa, synthetic construct
  REGION 1..8: note = Part sequence of HCDR1
GYTFTSYY

SEQ ID NO: 61 - protein, 8 aa, synthetic construct
  REGION 1..8: note = Part sequence of HCDR1
GYTFTTYW

SEQ ID NO: 62 - protein, 8 aa, synthetic construct
  REGION 1..8: note = Part sequence of HCDR1
GFDFSRYW

SEQ ID NO: 63 - protein, 8 aa, synthetic construct
  REGION 1..8: note = Part sequence of HCDR1
GYSFTSYW

SEQ ID NO: 64 - protein, 8 aa, synthetic construct
  REGION 1..8: note = Part sequence of HCDR1
GYTFTNFG

SEQ ID NO: 65 - protein, 8 aa, synthetic construct
  REGION 1..8: note = Part sequence of HCDR1
GYTFTNYG

SEQ ID NO: 66 - protein, 8 aa, synthetic construct
  REGION 1..8: note = Part sequence of HCDR1
GYIFTNYG

SEQ ID NO: 67 - protein, 8 aa, synthetic construct
  REGION 1..8: note = Part sequence of HCDR1
GYTFTDHT

SEQ ID NO: 68 - protein, 8 aa, synthetic construct
  REGION 1..8: note = Part sequence of HCDR1
GYSFTNYG

SEQ ID NO: 69 - protein, 8 aa, synthetic construct
  REGION 1..8: note = Part sequence of HCDR1
GYIFRNYG

SEQ ID NO: 70 - protein, 8 aa, synthetic construct
  REGION 1..8: note = Part sequence of HCDR1
GFTFTNYG

SEQ ID NO: 71 - protein, 8 aa, synthetic construct
  REGION 1..8: note = Part sequence of HCDR1
GYTFTDYG

SEQ ID NO: 72 - protein, 8 aa, synthetic construct
  REGION 1..8: note = Part sequence of HCDR2
GYSLTKYG

SEQ ID NO: 73 - protein, 8 aa, synthetic construct
  REGION 1..8: note = Part sequence of HCDR2
ISARSGST

SEQ ID NO: 74 - protein, 8 aa, synthetic construct
  REGION 1..8: note = Part sequence of HCDR2
IRYDGGST

SEQ ID NO: 75 - protein, 8 aa, synthetic construct
  REGION 1..8: note = Part sequence of HCDR2
ISYDGSRT

SEQ ID NO: 76 - protein, 8 aa, synthetic construct
  REGION 1..8: note = Part sequence of HCDR2
ISYDGSGT

SEQ ID NO: 77 - protein, 8 aa, synthetic construct
  REGION 1..8: note = Part sequence of HCDR2
LSYDGSGT

SEQ ID NO: 78 - protein, 8 aa, synthetic construct
  REGION 1..8: note = Part sequence of HCDR2
ISYDGIRT

SEQ ID NO: 79 - protein, 8 aa, synthetic construct
  REGION 1..8: note = Part sequence of HCDR2
ISYDGSNT

SEQ ID NO: 80 - protein, 8 aa, synthetic construct
  REGION 1..8: note = Part sequence of HCDR2
IKYDGSYT

SEQ ID NO: 81 - protein, 8 aa, synthetic construct
  REGION 1..8: note = Part sequence of HCDR2
ITNGGGST

SEQ ID NO: 82 - protein, 8 aa, synthetic construct
  REGION 1..8: note = Part sequence of HCDR2
LTNGGGST

SEQ ID NO: 83 - protein, 8 aa, synthetic construct
  REGION 1..8: note = Part sequence of HCDR2
LTDGGGST

SEQ ID NO: 84 - protein, 8 aa, synthetic construct
  REGION 1..8: note = Part sequence of HCDR2
IGPTNGVT

SEQ ID NO: 85 - protein, 8 aa, synthetic construct
  REGION 1..8: note = Part sequence of HCDR2
IGPTKGVT

SEQ ID NO: 86 - protein, 8 aa, synthetic construct
  REGION 1..8: note = Part sequence of HCDR2
ISIRGGST

SEQ ID NO: 87 - protein, 8 aa, synthetic construct
  REGION 1..8: note = Part sequence of HCDR2
ISTRGGST

SEQ ID NO: 88 - protein, 8 aa, synthetic construct
  REGION 1..8: note = Part sequence of HCDR2
ISTSGGST

SEQ ID NO: 89 - protein, 8 aa, synthetic construct
  REGION 1..8: note = Part sequence of HCDR2
IYPGDGDT

SEQ ID NO: 90 - protein, 8 aa, synthetic construct
  REGION 1..8: note = Part sequence of HCDR2
ITTSGGNT

SEQ ID NO: 91 - protein, 8 aa, synthetic construct
  REGION 1..8: note = Part sequence of HCDR2
ITTRGGST

SEQ ID NO: 92 - protein, 8 aa, synthetic construct
  REGION 1..8: note = Part sequence of HCDR2
ITFDGGRT

SEQ ID NO: 93 - protein, 8 aa, synthetic construct
  REGION 1..8: note = Part sequence of HCDR2
ISWGGRSI

SEQ ID NO: 94 - protein, 8 aa, synthetic construct
  REGION 1..8: note = Part sequence of HCDR2
ISYDGGST

SEQ ID NO: 95 - protein, 8 aa, synthetic construct
  REGION 1..8: note = Part sequence of HCDR2
INPNSGYT

SEQ ID NO: 96 - protein, 8 aa, synthetic construct
  REGION 1..8: note = Part sequence of HCDR2
INTRSGGT

SEQ ID NO: 97 - protein, 8 aa, synthetic construct
  REGION 1..8: note = Part sequence of HCDR2
INPSSGCS

SEQ ID NO: 98 - protein, 8 aa, synthetic construct
  REGION 1..8: note = Part sequence of HCDR2
IRPSSGYT

SEQ ID NO: 99 - protein, 8 aa, synthetic construct
  REGION 1..8: note = Part sequence of HCDR2
INTETGEP

SEQ ID NO: 100 - protein, 8 aa, synthetic construct
  REGION 1..8: note = Part sequence of HCDR2
INPSSGGT

SEQ ID NO: 101 - protein, 8 aa, synthetic construct
  REGION 1..8: note = Part sequence of HCDR2
INPSNGGT

SEQ ID NO: 102 - protein, 8 aa, synthetic construct
  REGION 1..8: note = Part sequence of HCDR2
INPGDGDT

SEQ ID NO: 103 - protein, 8 aa, synthetic construct
  REGION 1..8: note = Part sequence of HCDR2
INPDSSTI

SEQ ID NO: 104 - protein, 8 aa, synthetic construct
  REGION 1..8: note = Part sequence of HCDR2
IHPGNSDA

SEQ ID NO: 105 - protein, 8 aa, synthetic construct
  REGION 1..8: note = Part sequence of HCDR2
INTYTGEP

SEQ ID NO: 106 - protein, 8 aa, synthetic construct
  REGION 1..8: note = Part sequence of HCDR2
INTYAGEP

SEQ ID NO: 107 - protein, 8 aa, synthetic construct
  REGION 1..8: note = Part sequence of HCDR2
IFPNNGGT

SEQ ID NO: 108 - protein, 8 aa, synthetic construct
  REGION 1..8: note = Part sequence of HCDR2
LNTYTGEP

SEQ ID NO: 109 - protein, 8 aa, synthetic construct
  REGION 1..8: note = Part sequence of HCDR2
INTYTGQP

SEQ ID NO: 110 - protein, 8 aa, synthetic construct
  REGION 1..8: note = Part sequence of HCDR2
INTYTREP

SEQ ID NO: 111 - protein, 8 aa, synthetic construct
  REGION 1..8: note = Part sequence of HCDR2
INTYTGKP

SEQ ID NO: 112 - protein, 8 aa, synthetic construct
  REGION 1..8: note = Part sequence of HCDR2
INTYTGDP

SEQ ID NO: 113 - protein, 8 aa, synthetic construct
  REGION 1..8: note = Part sequence of HCDR2
INTYNGEP

SEQ ID NO: 114 - protein, 8 aa, synthetic construct
  REGION 1..8: note = Part sequence of HCDR2
INTYSGEP

SEQ ID NO: 115 - protein, 8 aa, synthetic construct
  REGION 1..8: note = Part sequence of HCDR3
ARGAFFDY

SEQ ID NO: 116 - protein, 9 aa, synthetic construct
  REGION 1..9: note = Part sequence of HCDR3
TTGYGSTGY

SEQ ID NO: 117 - protein, 19 aa, synthetic construct
  REGION 1..19: note = Part sequence of HCDR3
ARPYYYDGSYYRYYWFFDF

SEQ ID NO: 118 - protein, 13 aa, synthetic construct
  REGION 1..13: note = Part sequence of HCDR3
ARGGIIRGTLFDY

SEQ ID NO: 119 - protein, 13 aa, synthetic construct
  REGION 1..13: note = Part sequence of HCDR3
ARPFYNNYYWYDF

SEQ ID NO: 120 - protein, 18 aa, synthetic construct
  REGION 1..18: note = Part sequence of HCDR3
ARHGHYDGNYNYGGHFDY

SEQ ID NO: 121 - protein, 18 aa, synthetic construct
  REGION 1..18: note = Part sequence of HCDR3
ARHGFYDGNYYYGGSFDY

SEQ ID NO: 122 - protein, 13 aa, synthetic construct
  REGION 1..13: note = Part sequence of HCDR3
ARPYSNRYWYFDF

SEQ ID NO: 123 - protein, 9 aa, synthetic construct
  REGION 1..9: note = Part sequence of HCDR3
TRGNSAGDY

SEQ ID NO: 124 - protein, 11 aa, synthetic construct
  REGION 1..11: note = Part sequence of HCDR3
TRDRGHWVFDY

SEQ ID NO: 125 - protein, 11 aa, synthetic construct
  REGION 1..11: note = Part sequence of HCDR3
SRDRGHWVFDY

SEQ ID NO: 126 - protein, 16 aa, synthetic construct
  REGION 1..16: note = Part sequence of HCDR3
AREGDYGGYSEGPFDY

SEQ ID NO: 127 - protein, 6 aa, synthetic construct
  REGION 1..6: note = Part sequence of HCDR3
TTGFAY

SEQ ID NO: 128 - protein, 15 aa, synthetic construct
  REGION 1..15: note = Part sequence of HCDR3
ASRSGHNNYEGWFAY

SEQ ID NO: 129 - protein, 8 aa, synthetic construct
  REGION 1..8: note = Part sequence of HCDR3
SRHRYNYH

SEQ ID NO: 130 - protein, 8 aa, synthetic construct
  REGION 1..8: note = Part sequence of HCDR3
TRGRYNSR

SEQ ID NO: 131 - protein, 9 aa, synthetic construct
  REGION 1..9: note = Part sequence of HCDR3
ARHGRRLDY

SEQ ID NO: 132 - protein, 9 aa, synthetic construct
  REGION 1..9: note = Part sequence of HCDR3
ARHGRYLAS

SEQ ID NO: 133 - protein, 7 aa, synthetic construct
  REGION 1..7: note = Part sequence of HCDR3
TTGRLTR

SEQ ID NO: 134 - protein, 8 aa, synthetic construct
  REGION 1..8: note = Part sequence of HCDR3
ARHRNFAY

SEQ ID NO: 135 - protein, 8 aa, synthetic construct
  REGION 1..8: note = Part sequence of HCDR3
TRHRYLHL

SEQ ID NO: 136 - protein, 13 aa, synthetic construct
  REGION 1..13: note = Part sequence of HCDR3
TRVGGGPYWSFDF

SEQ ID NO: 137 - protein, 5 aa, synthetic construct
  REGION 1..5: note = Part sequence of HCDR3
TTKLG

SEQ ID NO: 138 - protein, 7 aa, synthetic construct
  REGION 1..7: note = Part sequence of HCDR3
TTGSFDY

SEQ ID NO: 139 - protein, 7 aa, synthetic construct
  REGION 1..7: note = Part sequence of HCDR3
ARSTFDY

SEQ ID NO: 140 - protein, 11 aa, synthetic construct
  REGION 1..11: note = Part sequence of HCDR3
AVYDGYFPFEY

SEQ ID NO: 141 - protein, 11 aa, synthetic construct
  REGION 1..11: note = Part sequence of HCDR3
SVYDDYFPFDY

SEQ ID NO: 142 - protein, 11 aa, synthetic construct
  REGION 1..11: note = Part sequence of HCDR3
AVFDGYFPFDY

SEQ ID NO: 143 - protein, 11 aa, synthetic construct
  REGION 1..11: note = Part sequence of HCDR3
AGYSKDYPLDY

SEQ ID NO: 144 - protein, 11 aa, synthetic construct
  REGION 1..11: note = Part sequence of HCDR3
AGYAKDYPMDY

SEQ ID NO: 145 - protein, 11 aa, synthetic construct
  REGION 1..11: note = Part sequence of HCDR3
AGFHKRYPMDY

SEQ ID NO: 146 - protein, 11 aa, synthetic construct
  REGION 1..11: note = Part sequence of HCDR3
VYGNYRYPMDY

SEQ ID NO: 147 - protein, 16 aa, synthetic construct
  REGION 1..16: note = Part sequence of HCDR3
VRPPHFYGSSLYAMDY

SEQ ID NO: 148 - protein, 15 aa, synthetic construct
  REGION 1..15: note = Part sequence of HCDR3
AREPHYYGNSYVRGY

SEQ ID NO: 149 - protein, 15 aa, synthetic construct
  REGION 1..15: note = Part sequence of HCDR3
AREPHYYGSSYVRGY

SEQ ID NO: 150 - protein, 13 aa, synthetic construct
  REGION 1..13: note = Part sequence of HCDR3
TRPPYYDYDEGDY

SEQ ID NO: 151 - protein, 16 aa, synthetic construct
  REGION 1..16: note = Part sequence of HCDR3
ARRGVYNYDVGTWFPY

SEQ ID NO: 152 - protein, 13 aa, synthetic construct
  REGION 1..13: note = Part sequence of HCDR3
ARWLRPDYYAMDY

SEQ ID NO: 153 - protein, 17 aa, synthetic construct
  REGION 1..17: note = Part sequence of HCDR3
ARRGFHYSNYAMAWFGY

SEQ ID NO: 154 - protein, 17 aa, synthetic construct
  REGION 1..17: note = Part sequence of HCDR3
ARRGYYGSYDPRTWFAY

SEQ ID NO: 155 - protein, 17 aa, synthetic construct
  REGION 1..17: note = Part sequence of HCDR3
TRRGFYGSHDPRTWFAY

SEQ ID NO: 156 - protein, 16 aa, synthetic construct
  REGION 1..16: note = Part sequence of HCDR3
ARRGVYNYDVGTWFAY

SEQ ID NO: 157 - protein, 8 aa, synthetic construct
  REGION 1..8: note = Part sequence of HCDR3
ARSGGFAY

SEQ ID NO: 158 - protein, 16 aa, synthetic construct
  REGION 1..16: note = Part sequence of HCDR3
ARRGGSYRYDGAWFVY

SEQ ID NO: 159 - protein, 11 aa, synthetic construct
  REGION 1..11: note = Part sequence of HCDR3
ARNYYGISGDY

SEQ ID NO: 160 - protein, 11 aa, synthetic construct
  REGION 1..11: note = Part sequence of HCDR3
GRNYYGISGDY

SEQ ID NO: 161 - protein, 11 aa, synthetic construct
  REGION 1..11: note = Part sequence of HCDR3
ARNHYERAMDY

SEQ ID NO: 162 - protein, 11 aa, synthetic construct
  REGION 1..11: note = Part sequence of HCDR3
ARNHYERGMDY

SEQ ID NO: 163 - protein, 11 aa, synthetic construct
  REGION 1..11: note = Part sequence of HCDR3
ARNHYERSMDY

SEQ ID NO: 164 - protein, 11 aa, synthetic construct
  REGION 1..11: note = Part sequence of LCDR1
QSLLHSSGNTY

SEQ ID NO: 165 - protein, 6 aa, synthetic construct
  REGION 1..6: note = Part sequence of LCDR1
KSISKY

SEQ ID NO: 166 - protein, 5 aa, synthetic construct
  REGION 1..5: note = Part sequence of LCDR1
SSVRY

SEQ ID NO: 167 - protein, 11 aa, synthetic construct
  REGION 1..11: note = Part sequence of LCDR1
KSLLYSNGKTY

SEQ ID NO: 168 - protein, 6 aa, synthetic construct
  REGION 1..6: note = Part sequence of LCDR1
QNINNY

SEQ ID NO: 169 - protein, 10 aa, synthetic construct
  REGION 1..10: note = Part sequence of LCDR1
QNVDYYGNSY

SEQ ID NO: 170 - protein, 11 aa, synthetic construct
  REGION 1..11: note = Part sequence of LCDR1
QSLVYSDGKTY

SEQ ID NO: 171 - protein, 6 aa, synthetic construct
  REGION 1..6: note = Part sequence of LCDR1
QNINRY

SEQ ID NO: 172 - protein, 6 aa, synthetic construct
  REGION 1..6: note = Part sequence of LCDR1
QNIDKY

SEQ ID NO: 173 - protein, 6 aa, synthetic construct
  REGION 1..6: note = Part sequence of LCDR1
QDIGNY

SEQ ID NO: 174 - protein, 11 aa, synthetic construct
  REGION 1..11: note = Part sequence of LCDR1
QSLLGTSGKTF

SEQ ID NO: 175 - protein, 11 aa, synthetic construct
  REGION 1..11: note = Part sequence of LCDR1
QSLLDNDGNTY

SEQ ID NO: 176 - protein, 12 aa, synthetic construct
  REGION 1..12: note = Part sequence of LCDR1
QSLLNSRTRNNY

SEQ ID NO: 177 - protein, 12 aa, synthetic construct
  REGION 1..12: note = Part sequence of LCDR1
QSLFNSRTRKNY

SEQ ID NO: 178 - protein, 12 aa, synthetic construct
  REGION 1..12: note = Part sequence of LCDR1
QSLLNRGNQKNY

SEQ ID NO: 179 - protein, 12 aa, synthetic construct
  REGION 1..12: note = Part sequence of LCDR1
QSLLNSGNRKNY

SEQ ID NO: 180 - protein, 12 aa, synthetic construct
  REGION 1..12: note = Part sequence of LCDR1
QSLLNSGKQKNY

SEQ ID NO: 181 - protein, 12 aa, synthetic construct
  REGION 1..12: note = Part sequence of LCDR1
QSLLNSRKQKNY

SEQ ID NO: 182 - protein, 11 aa, synthetic construct
  REGION 1..11: note = Part sequence of LCDR1
QSIVHSNGNTY

SEQ ID NO: 183 - protein, 5 aa, synthetic construct
  REGION 1..5: note = Part sequence of LCDR1
SSVNY

SEQ ID NO: 184 - protein, 10 aa, synthetic construct
  REGION 1..10: note = Part sequence of LCDR1
KSVSTSGYSY

SEQ ID NO: 185 - protein, 11 aa, synthetic construct
  REGION 1..11: note = Part sequence of LCDR1
QSLLDSDGKTY

SEQ ID NO: 186 - protein, 11 aa, synthetic construct
  REGION 1..11: note = Part sequence of LCDR1
QSLVHSNGNTY

SEQ ID NO: 187 - protein, 11 aa, synthetic construct
  REGION 1..11: note = Part sequence of LCDR1
QTLVHSNGNTY

SEQ ID NO: 188 - protein, 11 aa, synthetic construct
  REGION 1..11: note = Part sequence of LCDR1
QTLLHSNGNTY

SEQ ID NO: 189 - protein, 11 aa, synthetic construct
  REGION 1..11: note = Part sequence of LCDR1
HGLVHSNGNTY

SEQ ID NO: 190 - protein, 11 aa, synthetic construct
  REGION 1..11: note = Part sequence of LCDR1
QGLVHSNGNTY

SEQ ID NO: 191 - protein, 11 aa, synthetic construct
  REGION 1..11: note = Part sequence of LCDR1
QSLLHSNGNTY

SEQ ID NO: 192 - protein, 11 aa, synthetic construct
  REGION 1..11: note = Part sequence of LCDR1
QSLVHINGNTY

SEQ ID NO: 193 - protein, 9 aa, synthetic construct
  REGION 1..9: note = Part sequence of LCDR3
VQSTHAPWT

SEQ ID NO: 194 - protein, 10 aa, synthetic construct
  REGION 1..10: note = Part sequence of LCDR3
VQGTHAPPWT

SEQ ID NO: 195 - protein, 9 aa, synthetic construct
  REGION 1..9: note = Part sequence of LCDR3
QQHNEYPPT

SEQ ID NO: 196 - protein, 8 aa, synthetic construct
  REGION 1..8: note = Part sequence of LCDR3
HHHYSGYT

SEQ ID NO: 197 - protein, 8 aa, synthetic construct
  REGION 1..8: note = Part sequence of LCDR3
FQHNSGNT

SEQ ID NO: 198 - protein, 9 aa, synthetic construct
  REGION 1..9: note = Part sequence of LCDR3
QQWSNSPYT

SEQ ID NO: 199 - protein, 9 aa, synthetic construct
  REGION 1..9: note = Part sequence of LCDR3
QQWSSAPYT

SEQ ID NO: 200 - protein, 9 aa, synthetic construct
  REGION 1..9: note = Part sequence of LCDR3
QQFLEYPLT

SEQ ID NO: 201 - protein, 8 aa, synthetic construct
  REGION 1..8: note = Part sequence of LCDR3
QQYNSWIT

SEQ ID NO: 202 - protein, 8 aa, synthetic construct
  REGION 1..8: note = Part sequence of LCDR3
QQYNTWIT

SEQ ID NO: 203 - protein, 9 aa, synthetic construct
  REGION 1..9: note = Part sequence of LCDR3
QQGRRLPYT

SEQ ID NO: 204 - protein, 9 aa, synthetic construct
  REGION 1..9: note = Part sequence of LCDR3
VQTTHFPLT

SEQ ID NO: 205 - protein, 9 aa, synthetic construct
  REGION 1..9: note = Part sequence of LCDR3
FQHDTWPLT

SEQ ID NO: 206 - protein, 9 aa, synthetic construct
  REGION 1..9: note = Part sequence of LCDR3
FQHNSWPVT

SEQ ID NO: 207 - protein, 9 aa, synthetic construct
  REGION 1..9: note = Part sequence of LCDR3
LQHDSWPLT

SEQ ID NO: 208 - protein, 9 aa, synthetic construct
  REGION 1..9: note = Part sequence of LCDR3
LQHKQYPPT

SEQ ID NO: 209 - protein, 9 aa, synthetic construct
  REGION 1..9: note = Part sequence of LCDR3
WQGTHFPDT

SEQ ID NO: 210 - protein, 9 aa, synthetic construct
  REGION 1..9: note = Part sequence of LCDR3
VQARHFPFT

SEQ ID NO: 211 - protein, 9 aa, synthetic construct
  REGION 1..9: note = Part sequence of LCDR3
MQANHAPLT

SEQ ID NO: 212 - protein, 9 aa, synthetic construct
  REGION 1..9: note = Part sequence of LCDR3
KQSYNLPWT

SEQ ID NO: 213 - protein, 9 aa, synthetic construct
  REGION 1..9: note = Part sequence of LCDR3
QHSYNLPWT

SEQ ID NO: 214 - protein, 9 aa, synthetic construct
  REGION 1..9: note = Part sequence of LCDR3
QNDYSYPFT

SEQ ID NO: 215 - protein, 9 aa, synthetic construct
  REGION 1..9: note = Part sequence of LCDR3
QNDYSYPLT

SEQ ID NO: 216 - protein, 9 aa, synthetic construct
  REGION 1..9: note = Part sequence of LCDR3
QNEYSYPLT

SEQ ID NO: 217 - protein, 9 aa, synthetic construct
  REGION 1..9: note = Part sequence of LCDR3
FQGSHVPFT

SEQ ID NO: 218 - protein, 8 aa, synthetic construct
  REGION 1..8: note = Part sequence of LCDR3
HQWSSHPH

SEQ ID NO: 219 - protein, 8 aa, synthetic construct
  REGION 1..8: note = Part sequence of LCDR3
QHIRELTR

SEQ ID NO: 220 - protein, 8 aa, synthetic construct
  REGION 1..8: note = Part sequence of LCDR3
WQGTHFIH

SEQ ID NO: 221 - protein, 9 aa, synthetic construct
  REGION 1..9: note = Part sequence of LCDR3
SQSTHVPYT

SEQ ID NO: 222 - protein, 9 aa, synthetic construct
  REGION 1..9: note = Part sequence of LCDR3
SQSTQVPYT

SEQ ID NO: 223 - protein, 9 aa, synthetic construct
  REGION 1..9: note = Part sequence of LCDR3
SQSTLVPYT

SEQ ID NO: 224 - protein, 9 aa, synthetic construct
  REGION 1..9: note = Part sequence of LCDR3
SQSTHIPYT

SEQ ID NO: 225 - protein, 9 aa, synthetic construct
  REGION 1..9: note = Part sequence of LCDR3
SQSTHLPYT

SEQ ID NO: 226 - protein, 9 aa, synthetic construct
  REGION 1..9: note = Part sequence of LCDR3
SQSAHVPWT

SEQ ID NO: 227 - protein, 9 aa, synthetic construct
  REGION 1..9: note = Part sequence of LCDR3
SQSTHVPWT